European Patent Specification EP 4 444 357 B1, published May 21, 2025. Title: PLEASE ADD. Applicant: Please add. Application WO. The sequence listing filed with the application follows.

SEQUENCE LISTING (19 sequences)

SEQ ID NO: 1 - DNA, 24 bp, synthetic construct
  source 1..24: mol_type = other DNA
  misc_feature 24: note = 3'-O attached to a GalNAc-comprising compound via a linker
tttttttttttttttttttttttt

SEQ ID NO: 2 - DNA, 24 bp, synthetic construct
  source 1..24: mol_type = other DNA
  misc_feature 24: note = 3'-O attached to a GalNAc-comprising compound via a linker
  modified_base 2..24: mod_base = OTHER; note = 5'-thiophosphate
tttttttttttttttttttttttt

SEQ ID NO: 3 - DNA, 18 bp, synthetic construct
  source 1..18: mol_type = other DNA
cgggtggatgctgagaac

SEQ ID NO: 4 - DNA, 21 bp, synthetic construct
  source 1..21: mol_type = other DNA
tgcttcccattgtcaatctcc

SEQ ID NO: 5 - DNA, 23 bp, synthetic construct
  source 1..23: mol_type = other DNA
agtgaggagctgcgtgagaccaa

SEQ ID NO: 6 - RNA, 21 nt, synthetic construct
  source 1..21: mol_type = other RNA
  modified_base 1: mod_base = OTHER; note = 2'-O-methyl guanosine
  modified_base 2: mod_base = OTHER; note = 2'-fluoro cytidine 5'-thiophosphate
  modified_base 3: mod_base = OTHER; note = 2'-O-methyl guanosine 5'-thiophosphate
  modified_base 4: mod_base = OTHER; note = 2'-O-methyl uridine
  modified_base 5: mod_base = OTHER; note = 2'-fluoro cytidine
  modified_base 6: mod_base = OTHER; note = 2'-O-methyl adenosine
  modified_base 7: mod_base = OTHER; note = 2'-fluoro cytidine
  modified_base 8: mod_base = OTHER; note = 2'-O-methyl cytidine
  modified_base 9: mod_base = OTHER; note = 2'-fluoro adenosine
  modified_base 10: mod_base = OTHER; note = 2'-fluoro adenosine
  modified_base 11: mod_base = OTHER; note = 2'-O-methyl adenosine
  modified_base 12: mod_base = OTHER; note = 2'-O-methyl adenosine
  modified_base 13: mod_base = OTHER; note = 2'-fluoro adenosine
  modified_base 14: mod_base = OTHER; note = 2'-O-methyl guanosine
  modified_base 15: mod_base = OTHER; note = 2'-fluoro cytidine
  modified_base 16: mod_base = OTHER; note = 2'-O-methyl guanosine
  modified_base 17: mod_base = OTHER; note = 2'-O-methyl cytidine
  modified_base 18: mod_base = OTHER; note = 2'-fluoro adenosine
  modified_base 19: mod_base = OTHER; note = 2'-O-methyl adenosine
  modified_base 20: mod_base = OTHER; note = 2'-deoxy thymidine 5'-thiophosphate
  modified_base 21: mod_base = OTHER; note = 2'-deoxy thymidine 5'-thiophosphate
  misc_feature 21: note = 3'-O attached to a GalNAc-comprising compound via a linker
gcgtcaccaaaaagcgcaatt

SEQ ID NO: 7 - RNA, 21 nt, synthetic construct
  source 1..21: mol_type = other RNA
  modified_base 1: mod_base = OTHER; note = 2'-O-methyl uridine
  modified_base 2: mod_base = OTHER; note = 2'-deoxy thymidine 5'-thiophosphate
  modified_base 3: mod_base = OTHER; note = 2'-O-methyl guanosine 5'-thiophosphate
  modified_base 4: mod_base = OTHER; note = 2'-fluoro cytidine
  modified_base 5: mod_base = OTHER; note = 2'-O-methyl guanosine
  modified_base 6: mod_base = OTHER; note = 2'-fluoro cytidine
  modified_base 7: mod_base = OTHER; note = 2'-deoxy thymidine
  modified_base 8: mod_base = OTHER; note = 2'-O-methyl uridine 5'-thiophosphate
  modified_base 9: mod_base = OTHER; note = 2'-fluoro uridine
  modified_base 10: mod_base = OTHER; note = 2'-O-methyl uridine
  modified_base 11: mod_base = OTHER; note = 2'-O-methyl uridine
  modified_base 12: mod_base = OTHER; note = 2'-fluoro guanosine
  modified_base 13: mod_base = OTHER; note = 2'-O-methyl guanosine
  modified_base 14: mod_base = OTHER; note = 2'-fluoro uridine
  modified_base 15: mod_base = OTHER; note = 2'-O-methyl guanosine
  modified_base 16: mod_base = OTHER; note = 2'-fluoro adenosine
  modified_base 17: mod_base = OTHER; note = 2'-O-methyl cytidine
  modified_base 18: mod_base = OTHER; note = 2'-O-methyl guanosine
  modified_base 20: mod_base = OTHER; note = 2'-O-methyl uridine 5'-thiophosphate
  modified_base 21: mod_base = OTHER; note = 2'-O-methyl uridine 5'-thiophosphate
  modified_base 19: mod_base = OTHER; note = 2'-deoxy cytidine
ttgcgctttttggtgacgctt

SEQ ID NO: 8 - DNA, 22 bp, synthetic construct
  source 1..22: mol_type = other DNA
ggaccaggtggaacagtataag

SEQ ID NO: 9 - DNA, 20 bp, synthetic construct
  source 1..20: mol_type = other DNA
tcaatgcggattcgagactg

SEQ ID NO: 10 - DNA, 28 bp, synthetic construct
  source 1..28: mol_type = other DNA
  misc_feature 1: note = 5'-fluorophore
  misc_feature 10: note = ZEN TM quencher
  misc_feature 28: note = 3'-Iowa BlackTM FQ (IBFQ) quencher
cagcttggcggagtatgtcttttctagc

SEQ ID NO: 11 - RNA, 21 nt, synthetic construct
  source 1..21: mol_type = other RNA
  modified_base 1: mod_base = OTHER; note = 2'-O-methyl uridine
  modified_base 2: mod_base = OTHER; note = 2'-fluoro guanosine 5'-thiophosphate
  modified_base 3: mod_base = OTHER; note = 2'-O-methyl adenosine 5'-thiophosphate
  modified_base 4: mod_base = OTHER; note = 2'-O-methyl cytidine
  modified_base 5: mod_base = OTHER; note = 2'-O-methyl uridine
  modified_base 6: mod_base = OTHER; note = 2'-fluoro uridine
  modified_base 7: mod_base = OTHER; note = 2'-O-methyl uridine
  modified_base 8: mod_base = OTHER; note = 2'-fluoro guanosine
  modified_base 9: mod_base = OTHER; note = 2'-fluoro cytidine
  modified_base 10: mod_base = OTHER; note = 2'-O-methyl adenosine
  modified_base 11: mod_base = OTHER; note = 2'-O-methyl uridine
  modified_base 12: mod_base = OTHER; note = 2'-O-methyl uridine
  modified_base 13: mod_base = OTHER; note = 2'-O-methyl cytidine
  modified_base 14: mod_base = OTHER; note = 2'-fluoro cytidine
  modified_base 15: mod_base = OTHER; note = 2'-O-methyl adenosine
  modified_base 16: mod_base = OTHER; note = 2'-fluoro guanosine
  modified_base 17: mod_base = OTHER; note = 2'-O-methyl adenosine
  modified_base 18: mod_base = OTHER; note = 2'-O-methyl cytidine
  modified_base 19: mod_base = OTHER; note = 2'-O-methyl cytidine
  modified_base 20: mod_base = OTHER; note = 2'-deoxy thymidine 5'-thiophosphate
  modified_base 21: mod_base = OTHER; note = 2'-deoxy thymidine 5'-thiophosphate
tgactttgcattccagacctt

SEQ ID NO: 12 - RNA, 21 nt, synthetic construct
  source 1..21: mol_type = other RNA
  modified_base 1: mod_base = OTHER; note = 2'-O-methyl guanosine
  modified_base 2: mod_base = OTHER; note = 2'-O-methyl guanosine 5'-thiophosphate
  modified_base 3: mod_base = OTHER; note = 2'-O-methyl uridine 5'-thiophosphate
  modified_base 4: mod_base = OTHER; note = 2'-O-methyl cytidine
  modified_base 5: mod_base = OTHER; note = 2'-O-methyl uridine
  modified_base 6: mod_base = OTHER; note = 2'-O-methyl guanosine
  modified_base 7: mod_base = OTHER; note = 2'-fluoro guanosine
  modified_base 8: mod_base = OTHER; note = 2'-O-methyl adenosine
  modified_base 9: mod_base = OTHER; note = 2'-fluoro adenosine
  modified_base 10: mod_base = OTHER; note = 2'-fluoro uridine
  modified_base 11: mod_base = OTHER; note = 2'-fluoro guanosine
  modified_base 12: mod_base = OTHER; note = 2'-O-methyl cytidine
  modified_base 13: mod_base = OTHER; note = 2'-O-methyl adenosine
  modified_base 14: mod_base = OTHER; note = 2'-O-methyl adenosine
  modified_base 15: mod_base = OTHER; note = 2'-O-methyl adenosine
  modified_base 16: mod_base = OTHER; note = 2'-O-methyl guanosine
  modified_base 17: mod_base = OTHER; note = 2'-O-methyl uridine
  modified_base 18: mod_base = OTHER; note = 2'-O-methyl cytidine
  modified_base 19: mod_base = OTHER; note = 2'-O-methyl adenosine
  modified_base 20: mod_base = OTHER; note = 2'-deoxy thymidine 5'-thiophosphate
  modified_base 21: mod_base = OTHER; note = 2'-deoxy thymidine 5'-thiophosphate
  misc_feature 21: note = 3'-O attached to a GalNAc-comprising compound via a linker
ggtctggaatgcaaagtcatt

SEQ ID NO: 13 - DNA, 20 bp, synthetic construct
  source 1..20: mol_type = other DNA
tcaccaagatcctgcatgtc

SEQ ID NO: 14 - DNA, 18 bp, synthetic construct
  source 1..18: mol_type = other DNA
gttccacgggatgctctg

SEQ ID NO: 15 - DNA, 23 bp, synthetic construct
  source 1..23: mol_type = other DNA
  misc_feature 1: note = 5'-fluorophore
  misc_feature 10: note = ZEN TM quencher
  misc_feature 23: note = 3'-Iowa BlackTM FQ (IBFQ) quencher
caggtcgccactcatcttcacca

SEQ ID NO: 16 - RNA, 21 nt, synthetic construct
  source 1..21: mol_type = other RNA
  modified_base 20: mod_base = OTHER; note = 2'-deoxy thymidine
  modified_base 21: mod_base = OTHER; note = 2'-deoxy thymidine
gcgtcaccaaaaagcgcaatt

SEQ ID NO: 17 - RNA, 21 nt, synthetic construct
  source 1..21: mol_type = other RNA
  modified_base 2: mod_base = OTHER; note = 2'-deoxy thymidine
  modified_base 7: mod_base = OTHER; note = 2'-deoxy thymidine
ttgcgctttttggtgacgctt

SEQ ID NO: 18 - RNA, 21 nt, synthetic construct
  source 1..21: mol_type = other RNA
  modified_base 20: mod_base = OTHER; note = 2'-deoxy thymidine
  modified_base 21: mod_base = OTHER; note = 2'-deoxy thymidine
tgactttgcattccagacctt

SEQ ID NO: 19 - RNA, 21 nt, synthetic construct
  source 1..21: mol_type = other RNA
  modified_base 20: mod_base = OTHER; note = 2'-deoxy thymidine
  modified_base 21: mod_base = OTHER; note = 2'-deoxy thymidine
ggtctggaatgcaaagtcatt